European Patent Application EP 4 375 295 A1, published May 29, 2024. Title: 자가면역질환의 예방 또는 치료를 위한 항체의약품. Applicant: 주식회사 이뮨메드. The sequence listing filed with the application follows.

SEQUENCE LISTING (21 sequences)

SEQ ID NO: 1 - protein, 5 aa, Artificial Sequence
GYNMN

SEQ ID NO: 2 - protein, 17 aa, Artificial Sequence
NIDPYYGSDTYAQKFQG

SEQ ID NO: 3 - protein, 16 aa, Artificial Sequence
NIDPYYGSTTYAQKFQ

SEQ ID NO: 4 - protein, 9 aa, Artificial Sequence
ETGTRAMDY

SEQ ID NO: 5 - protein, 8 aa, Artificial Sequence
ETGNRAMD

SEQ ID NO: 6 - protein, 11 aa, Artificial Sequence
RASENIYSNLA

SEQ ID NO: 7 - protein, 7 aa, Artificial Sequence
VADNLAD

SEQ ID NO: 8 - protein, 7 aa, Artificial Sequence
VATNLAD

SEQ ID NO: 9 - protein, 7 aa, Artificial Sequence
VADNLGD

SEQ ID NO: 10 - protein, 7 aa, Artificial Sequence
VADNRGD

SEQ ID NO: 11 - protein, 9 aa, Artificial Sequence
QHFYGSPRT

SEQ ID NO: 12 - protein, 9 aa, Artificial Sequence
QHFYGTPRT

SEQ ID NO: 13 - protein, 30 aa, Artificial Sequence
EVQLVQSGAEVKKPGASVKVSCKASGYTFT

SEQ ID NO: 14 - protein, 14 aa, Artificial Sequence
WVRQAPGKGLEWMG

SEQ ID NO: 15 - protein, 32 aa, Artificial Sequence
RVTMTVDKSISTAYMELSRLRSDDTAVYYCAR

SEQ ID NO: 16 - protein, 11 aa, Artificial Sequence
WGQGTLVTVSS

SEQ ID NO: 17 - protein, 23 aa, Artificial Sequence
DIQMTQSPSSLSASVGDRVTITC

SEQ ID NO: 18 - protein, 15 aa, Artificial Sequence
WYQQKPGKAPKLLIY

SEQ ID NO: 19 - protein, 32 aa, Artificial Sequence
GVPSRFSGSGSGTDFTLTISSLQPEDFATYYC

SEQ ID NO: 20 - protein, 10 aa, Artificial Sequence
FGGGTKVEIK

SEQ ID NO: 21 - protein, 137 aa, Artificial Sequence
SRLGDLYEEEMRELRRQVDQLTNDKARVEVERDNLAEDIMRLREKLQEEMLQREEAENTLQSFRQDVDNASLARLDLERKVESLQEEIAFLKKLHEEEIQELQAQIQEQHVQIDVDVSKPDLTAALRDVRQQYESVA